European Patent Application EP 4 484 549 A1, published January 1, 2025. Title: 乳酸菌、乳酸菌組成物、乳酸菌の製造方法、乳酸菌の酸耐性向上方法、乳酸菌のスクリーニング方法、及び発酵乳の製造方法. Applicant: Meiji Co., Ltd. The sequence listing filed with the application follows.

SEQUENCE LISTING (7 sequences)

SEQ ID NO: 1 - protein, 676 aa, Lactobacillus delbrueckii
MEVENKLNRMTAAGLLIAIGIVYGDIGTSPLYVMKSVIAGNGGINTVGRDLIIGTISLILWTVTLLTTVQTVIIALRATNHGEGGIFALYALIRKKAAWLVWPALIGGAAILADGTLTPAVTVTTAIEGLKGLEFGKGNVPVSNQTTVLVITIVILLVLFSIQRMGTRIIGKAFGPIMLVWFAFLGVMGLINIGGNWWILQALNPYYAIKLLFSPYNKAGFAILGSIFLATTGAEALYSDVGHVGKGNIIGSWPFVFVCLSLNYFGQGVWILNNTNMHSATEINPFYAMIPENIRLVSIVLATLAAIIASQALITGSFTLVAESINLKFLPRMNILYPSDERGQIYIPAVNKMLGITTIALVLFFRTSAHMEAAYGLSITISMLTTTILLYEWLVLKQVHNLANLLFVIFFSTINILFMGSSLSKFTHGGYVSLLITLLIASVMVVWYFGNKVRDQNGAGNAYVRLDEYTDMLTDLSHDDNYPTYSDNLVYMANVKYNKFIKREILYSILDKRPKRARAYWFVTVNVTNEPFTAEYAVNTFGTKNVINIQLYLGFKKQTSVNVYLRQIVHDLIKDNTIEAQPQEYTTTPGRDVGDFKFVIVNDVISPSTTLSSYKKWLVKARVQLQNLSPNPAQWFGLEFADMVIERVPLILGKQEPERIKRVAPVDYSKTSLNKK

SEQ ID NO: 2 - DNA, 2031 bp, Lactobacillus delbrueckii
  source 1..2031: mol_type = genomic DNA
atggaagtagaaaataaactcaatcgcatgacggccgccggcctcttgatcgcgattgggattgtctacggcgacatcgggaccagtcccctgtatgtcatgaaatccgtaatcgccggcaacggcggcatcaatacggtcggccgtgacttgatcatcgggaccatttccttgatcctgtggaccgtgaccctgctcacgacggtgcagaccgtgattatcgccttgagggcaaccaaccacggcgaaggcggtatcttcgccctctacgccttgatcagaaagaaagcagcctggctggtctggccggccttgatcggcggggctgccatcctggccgacgggaccctgaccccggccgtgacggttaccaccgccattgaagggctgaagggtctggaatttggcaagggcaatgtcccggtcagcaaccagaccacggtcttagtcattactattgttattttgctggtgcttttctccatccagcggatggggaccagaatcatcggaaaggctttcggtccaatcatgcttgtctggttcgccttcctgggcgtcatgggcttgatcaacatcggcggcaactggtggatcctgcaggccttgaacccttactacgcgatcaaattgctctttagcccttacaacaaggcgggcttcgcgatcttagggtccatcttcctggccaccacgggggctgaagccctttactccgacgtcggccacgtcggcaagggtaacatcattggctcctggccatttgtttttgtctgcctctccctgaactacttcgggcaaggggtttggatcttaaacaacaccaacatgcactcagccactgaaatcaaccccttctatgccatgattccggaaaatatccggctggtatcaatcgttctggccaccctggcagcgatcatcgcttcccaggccttgatcacgggttccttcaccctggtggctgaatccatcaacctgaagttcctgccgcggatgaacatcctctacccatctgatgaaagagggcagatctacatcccggccgttaacaagatgctaggcattactactattgccctggttctcttcttcagaacctcagcccacatggaagcagcctacggtctgtcaatcacgatttccatgctgacgaccaccatcctgctctacgaatggctggtgctcaagcaggtccacaacctggccaacctgctcttcgtgatcttcttcagtactatcaacatcctcttcatgggttcaagtctgagcaagttcactcacggcggttacgtgtcactgttgatcaccctcttgatcgcttcagtcatggtcgtttggtacttcggcaacaaggtccgggatcaaaacggagccggcaatgcctatgtccgcttggatgaatacacggacatgctgaccgacctcagccacgacgacaactacccgacctactctgacaacctggtttacatggccaacgtcaagtacaacaagttcatcaagcgcgaaatcctctactcaattctggacaagcggccaaagcgggcccgggcttactggttcgtcacggtcaacgtgaccaacgagccgtttaccgctgaatacgcggtcaacacttttggcaccaagaatgtgatcaacatccagctctaccttggtttcaagaagcaaaccagcgttaacgtttacctgcgccagatcgtccacgacttgatcaaggacaacacgatcgaggcccagccacaggaatacacgactactcctggccgggacgtcggcgacttcaagttcgtcatcgtcaacgacgtcatctcaccttcgaccaccctgtcttcttacaagaagtggctggtcaaggcccgcgtccagctgcagaacctgtcgcctaacccggctcaatggttcggcctggaattcgcggacatggtcatcgaacgcgtgcctttgatccttggtaagcaagagcctgaaagaatcaagcgggttgctccggttgactacagtaagacctcgctgaacaagaagtaa

SEQ ID NO: 3 - protein, 227 aa, Lactobacillus delbrueckii
GNKVRDQNGAGNAYVRLDEYTDMLTDLSHDDNYPTYSDNLVYMANVKYNKFIKREILYSILDKRPKRARAYWFVTVNVTNEPFTAEYAVNTFGTKNVINIQLYLGFKKQTSVNVYLRQIVHDLIKDNTIEAQPQEYTTTPGRDVGDFKFVIVNDVISPSTTLSSYKKWLVKARVQLQNLSPNPAQWFGLEFADMVIERVPLILGKQEPERIKRVAPVDYSKTSLNKK

SEQ ID NO: 4 - DNA, 684 bp, Lactobacillus delbrueckii
  source 1..684: mol_type = genomic DNA
ggcaacaaggtccgggatcaaaacggagccggcaatgcctatgtccgcttggatgaatacacggacatgctgaccgacctcagccacgacgacaactacccgacctactctgacaacctggtttacatggccaacgtcaagtacaacaagttcatcaagcgcgaaatcctctactcaattctggacaagcggccaaagcgggcccgggcttactggttcgtcacggtcaacgtgaccaacgagccgtttaccgctgaatacgcggtcaacacttttggcaccaagaatgtgatcaacatccagctctaccttggtttcaagaagcaaaccagcgttaacgtttacctgcgccagatcgtccacgacttgatcaaggacaacacgatcgaggcccagccacaggaatacacgactactcctggccgggacgtcggcgacttcaagttcgtcatcgtcaacgacgtcatctcaccttcgaccaccctgtcttcttacaagaagtggctggtcaaggcccgcgtccagctgcagaacctgtcgcctaacccggctcaatggttcggcctggaattcgcggacatggtcatcgaacgcgtgcctttgatccttggtaagcaagagcctgaaagaatcaagcgggttgctccggttgactacagtaagacctcgctgaacaagaagtaa

SEQ ID NO: 5 - protein, 19 aa, Lactobacillus delbrueckii
KAFGPIMLVWFAFLGVMGL

SEQ ID NO: 6 - protein, 18 aa, synthetic construct
  REGION 1..18: note = strain_i-172-189a.a.
KASVQSCLSGSPSWASWA

SEQ ID NO: 7 - protein, 19 aa, synthetic construct
  REGION 1..19: note = strain_i-1-172-190a.a.
KGFGPIMLVWFAFLGVMGL